European Patent Application EP 4 173 638 A1, published May 3, 2023. Title: ANTI-CD70 ANTIBODY AND APPLICATION THEREOF. Applicant: Jiangsu Hengrui Medicine Co., Ltd. Shanghai Hengrui Pharmaceutical Co., Ltd. The sequence listing filed with the application follows.

SEQUENCE LISTING (84 sequences)

SEQ ID NO: 1 - protein, 191 aa, Artificial Sequence
  PEPTIDE: Sequence of His-tagged CD70 protein extracellular domain
HHHHHHACGCAAAPDIKDLLSRLEELEGLVSSLREQQRFAQAQQQLPLESLGWDVAELQLNHTGPQQDPRLYWQGGPALGRSFLHGPELDKGQLRIHRDGIYMVHIQVTLAICSSTTASRHHPTTLAVGICSPASRSISLLRLSFHQGCTIASQRLTPLARGDTLCTNLTGTLLPSRNTDETFFGVQWVRP

SEQ ID NO: 2 - protein, 387 aa, Artificial Sequence
  PEPTIDE: Sequence of fusion protein of CD70 protein extracellular domain and Human-IgG1-Fc
QRFAQAQQQLPLESLGWDVAELQLNHTGPQQDPRLYWQGGPALGRSFLHGPELDKGQLRIHRDGIYMVHIQVTLAICSSTTASRHHPTTLAVGICSPASRSISLLRLSFHQGCTIASQRLTPLARGDTLCTNLTGTLLPSRNTDETFFGVQWVRPEPKSSDKTHTCPPCPAPELLGGPSVFLFPPKPKDTLMISRTPEVTCVVVDVSHEDPEVKFNWYVDGVEVHNAKTKPREEQYNSTYRVVSVLTVLHQDWLNGKEYKCKVSNKALPAPIEKTISKAKGQPREPQVYTLPPSRDELTKNQVSLTCLVKGFYPSDIAVEWESNGQPENNYKTTPPVLDSDGSFFLYSKLTVDKSRWQQGNVFSCSVMHEALHNHYTQKSLSLSPGK

SEQ ID NO: 3 - protein, 119 aa, Artificial Sequence
  DOMAIN: Amino acid sequence of heavy chain variable region of B1
QVQMQQSGAELVKPGASVMMSCKASGYTFTTYNIHWIKQTPGQGLEWIGDIYPGNGDASYNQKFRDRATLTADRSSSTAYLQLSSLTSEDSAIYYCATFSRFDGWFAYWGQGTLVTVSA

SEQ ID NO: 4 - protein, 111 aa, Artificial Sequence
  DOMAIN: Amino acid sequence of light chain variable region of B1
DIVMSQSPASLAVSLGQRATISCRASRSVSTSGYSYMHWYQQKPGQPPKLLIYLASNLESGVPARFSGSGSGTNFTLNIHPVEEEDAATYYCQHSRELPYTFGGGTKLEIK

SEQ ID NO: 5 - protein, 120 aa, Artificial Sequence
  DOMAIN: Amino acid sequence of heavy chain variable region of B7
QIQLVQSGPELKKPGETVKISCKTSGYTFTNYGMNWVRQAPGKGLKWMGWINTYTGEPTYADDFKGRFAFSLETSAGTAYLQINNLENEDTATYFCARGDSFTTEILRNWYFDVWGAGTT

SEQ ID NO: 6 - protein, 107 aa, Artificial Sequence
  DOMAIN: Amino acid sequence of light chain variable region of B7
DIQMTQTPASLSASVGETVTITCGASENIYGALNWYQRKQGKSPQLLIYGATNLADGMSSRFSGSGSGRQYSLKISSLHPDDVATYYCQNVLSTPWTFGGGTKLEMK

SEQ ID NO: 7 - protein, 120 aa, Artificial Sequence
  DOMAIN: Amino acid sequence of heavy chain variable region of F4
QVQLKQSGAELVKPGASVKMSCKASGDTFPRYNMHWLKQTPGQGLEWIGAIFPGNGETSYNQNFKGKATLTADKSSSTAYMQLNSLTSEDSAVYYCARNSYYDYAWFTYWGQGTLVTVSA

SEQ ID NO: 8 - protein, 111 aa, Artificial Sequence
  DOMAIN: Amino acid sequence of light chain variable region of F4
DIVMTQSPASLDVSLGQRATISCRASKSVSSSGYSFMHWYQQKPGQPPKLLISLASNLESGVPARFSGSGSGTDFTLTIYPVEEEDAATYYCQHSREFPPTFGSGTKLEIK

SEQ ID NO: 9 - protein, 5 aa, Artificial Sequence
  DOMAIN: Amino acid sequence of HCDR1 of B1
TYNIH

SEQ ID NO: 10 - protein, 17 aa, Artificial Sequence
  DOMAIN: Amino acid sequence of HCDR2 of B1
DIYPGNGDASYNQKFRD

SEQ ID NO: 11 - protein, 10 aa, Artificial Sequence
  DOMAIN: Amino acid sequence of HCDR3 of B1
FSRFDGWFAY

SEQ ID NO: 12 - protein, 15 aa, Artificial Sequence
  DOMAIN: Amino acid sequence of LCDR1 of B1
RASRSVSTSGYSYMH

SEQ ID NO: 13 - protein, 7 aa, Artificial Sequence
  DOMAIN: Amino acid sequence of LCDR2 of B1 or F4
LASNLES

SEQ ID NO: 14 - protein, 9 aa, Artificial Sequence
  DOMAIN: Amino acid sequence of LCDR3 of B1
QHSRELPYT

SEQ ID NO: 15 - protein, 5 aa, Artificial Sequence
  DOMAIN: Amino acid sequence of HCDR1 of B7
NYGMN

SEQ ID NO: 16 - protein, 17 aa, Artificial Sequence
  DOMAIN: Amino acid sequence of HCDR2 of B7
WINTYTGEPTYADDFKG

SEQ ID NO: 17 - protein, 16 aa, Artificial Sequence
  DOMAIN: Amino acid sequence of HCDR3 of B7
GDSFTTEILRNWYFDV

SEQ ID NO: 18 - protein, 11 aa, Artificial Sequence
  DOMAIN: Amino acid sequence of LCDR1 of B7
GASENIYGALN

SEQ ID NO: 19 - protein, 7 aa, Artificial Sequence
  DOMAIN: Amino acid sequence of LCDR2 of B7
GATNLAD

SEQ ID NO: 20 - protein, 9 aa, Artificial Sequence
  DOMAIN: Amino acid sequence of LCDR3 of B7
QNVLSTPWT

SEQ ID NO: 21 - protein, 5 aa, Artificial Sequence
  DOMAIN: Amino acid sequence of HCDR1 of F4
RYNMH

SEQ ID NO: 22 - protein, 17 aa, Artificial Sequence
  DOMAIN: Amino acid sequence of HCDR2 of F4
AIFPGNGETSYNQNFKG

SEQ ID NO: 23 - protein, 11 aa, Artificial Sequence
  DOMAIN: Amino acid sequence of HCDR3 of F4
NSYYDYAWFTY

SEQ ID NO: 24 - protein, 15 aa, Artificial Sequence
  DOMAIN: Amino acid sequence of LCDR1 of F4
RASKSVSSSGYSFMH

SEQ ID NO: 25 - protein, 9 aa, Artificial Sequence
  DOMAIN: Amino acid sequence of LCDR3 of F4
QHSREFPPT

SEQ ID NO: 26 - protein, 119 aa, Artificial Sequence
  DOMAIN: Sequence of heavy chain variable region of huB1VH1
EVQLVQSGAEVKKPGASVKVSCKASGYTFTTYNIHWVRQAPGQGLEWMGDIYPGNGDASYNQKFRDRVTMTRDTSTSTVYMELSSLRSEDTAVYYCARFSRFDGWFAYWGQGTLVTVSS

SEQ ID NO: 27 - protein, 119 aa, Artificial Sequence
  DOMAIN: Sequence of heavy chain variable region of huB1VH2
EVQMVQSGAEVKKPGASVKVSCKASGYTFTTYNIHWVRQAPGQGLEWMGDIYPGNGDASYNQKFRDRVTMTRDTSTSTVYMELSSLRSEDTAVYYCATFSRFDGWFAYWGQGTLVTVSS

SEQ ID NO: 28 - protein, 119 aa, Artificial Sequence
  DOMAIN: Sequence of heavy chain variable region of huB1VH3
EVQMVQSGAEVKKPGASVKVSCKASGYTFTTYNIHWVRQAPGQGLEWMGDIYPGNGDASYNQKFRDRVTMTADRSTSTVYMELSSLRSEDTAVYYCATFSRFDGWFAYWGQGTLVTVSS

SEQ ID NO: 29 - protein, 119 aa, Artificial Sequence
  DOMAIN: Sequence of heavy chain variable region of huB1VH4
EVQMVQSGAEVKKPGASVKVSCKASGYTFTTYNIHWVRQAPGQGLEWMGDIYPGNGDASYNQKFRDRVTLTADRSTSTAYMELSSLRSEDTAVYYCATFSRFDGWFAYWGQGTLVTVSS

SEQ ID NO: 30 - protein, 119 aa, Artificial Sequence
  DOMAIN: Sequence of heavy chain variable region of huB1VH5
EVQMVQSGAEVKKPGASVKVSCKASGYTFTTYNIHWVRQAPGQGLEWIGDIYPGNGDASYNQKFRDRATLTADRSTSTAYLELSSLRSEDTAVYYCATFSRFDGWFAYWGQGTLVTVSS

SEQ ID NO: 31 - protein, 119 aa, Artificial Sequence
  DOMAIN: Sequence of heavy chain variable region of huB1VH6
EVQMVQSGAEVKKPGASVKVSCKASGYTFTTYNIHWIKQAPGQGLEWIGDIYPGNGDASYNQKFRDRATLTADRSTSTAYLELSSLRSEDTAVYYCATFSRFDGWFAYWGQGTLVTVSS

SEQ ID NO: 32 - protein, 111 aa, Artificial Sequence
  DOMAIN: Sequence of light chain variable region of huB1VL1
DIVMTQSPDSLAVSLGERATINCRASRSVSTSGYSYMHWYQQKPGQPPKLLIYLASNLESGVPDRFSGSGSGTDFTLTISSLQAEDVAVYYCQHSRELPYTFGGGTKVEIK

SEQ ID NO: 33 - protein, 111 aa, Artificial Sequence
  DOMAIN: Sequence of light chain variable region of huB1VL2
DIVMSQSPDSLAVSLGERATINCRASRSVSTSGYSYMHWYQQKPGQPPKLLIYLASNLESGVPDRFSGSGSGTNFTLTISSLQAEDVAVYYCQHSRELPYTFGGGTKVEIK

SEQ ID NO: 34 - protein, 119 aa, Artificial Sequence
  DOMAIN: Sequence of heavy chain variable region of huB1VH1-1
EVQLVQSGAEVKKPGASVKVSCKASGYTFTTYNIHWVRQAPGQGLEWMGDIYPGTGDASYNQKFRDRVTMTRDTSTSTVYMELSSLRSEDTAVYYCARFSRFDGWFAYWGQGTLVTVSS

SEQ ID NO: 35 - protein, 119 aa, Artificial Sequence
  DOMAIN: Sequence of heavy chain variable region of huB1VH2-1
EVQMVQSGAEVKKPGASVKVSCKASGYTFTTYNIHWVRQAPGQGLEWMGDIYPGTGDASYNQKFRDRVTMTRDTSTSTVYMELSSLRSEDTAVYYCATFSRFDGWFAYWGQGTLVTVSS

SEQ ID NO: 36 - protein, 119 aa, Artificial Sequence
  DOMAIN: Sequence of heavy chain variable region of huB1VH3-1
EVQMVQSGAEVKKPGASVKVSCKASGYTFTTYNIHWVRQAPGQGLEWMGDIYPGTGDASYNQKFRDRVTMTADRSTSTVYMELSSLRSEDTAVYYCATFSRFDGWFAYWGQGTLVTVSS

SEQ ID NO: 37 - protein, 119 aa, Artificial Sequence
  DOMAIN: Sequence of heavy chain variable region of huB1VH4-1
EVQMVQSGAEVKKPGASVKVSCKASGYTFTTYNIHWVRQAPGQGLEWMGDIYPGTGDASYNQKFRDRVTLTADRSTSTAYMELSSLRSEDTAVYYCATFSRFDGWFAYWGQGTLVTVSS

SEQ ID NO: 38 - protein, 119 aa, Artificial Sequence
  DOMAIN: Sequence of heavy chain variable region of huB1VH5-1
EVQMVQSGAEVKKPGASVKVSCKASGYTFTTYNIHWVRQAPGQGLEWIGDIYPGTGDASYNQKFRDRATLTADRSTSTAYLELSSLRSEDTAVYYCATFSRFDGWFAYWGQGTLVTVSS

SEQ ID NO: 39 - protein, 119 aa, Artificial Sequence
  DOMAIN: Sequence of heavy chain variable region of huB1VH6-1
EVQMVQSGAEVKKPGASVKVSCKASGYTFTTYNIHWIKQAPGQGLEWIGDIYPGTGDASYNQKFRDRATLTADRSTSTAYLELSSLRSEDTAVYYCATFSRFDGWFAYWGQGTLVTVSS

SEQ ID NO: 40 - protein, 111 aa, Artificial Sequence
  DOMAIN: Sequence of light chain variable region of huB1VL1-1
DIVMTQSPDSLAVSLGERATINCRASRSVSTSGYSYMHWYQQKPGQPPKLLIYLADNLESGVPDRFSGSGSGTDFTLTISSLQAEDVAVYYCQHSRELPYTFGGGTKVEIK

SEQ ID NO: 41 - protein, 111 aa, Artificial Sequence
  DOMAIN: Sequence of heavy chain variable region of huB1VL2-1
DIVMSQSPDSLAVSLGERATINCRASRSVSTSGYSYMHWYQQKPGQPPKLLIYLADNLESGVPDRFSGSGSGTNFTLTISSLQAEDVAVYYCQHSRELPYTFGGGTKVEIK

SEQ ID NO: 42 - protein, 17 aa, Artificial Sequence
  DOMAIN: Amino acid sequence of HCDR2 mutant of B1
DIYPGTGDASYNQKFRD

SEQ ID NO: 43 - protein, 7 aa, Artificial Sequence
  DOMAIN: Amino acid sequence of LCDR2 mutant of B1 or F4
LADNLES

SEQ ID NO: 44 - protein, 125 aa, Artificial Sequence
  DOMAIN: Amino acid sequence of heavy chain variable region of huB7VH1
EVQLVQSGSELKKPGASVKVSCKASGYTFTNYGMNWVRQAPGQGLEWMGWINTYTGEPTYADDFKGRFVFSLDTSVSTAYLQISSLKAEDTAVYYCARGDSFTTEILRNWYFDVWGQGTTVTVSS

SEQ ID NO: 45 - protein, 125 aa, Artificial Sequence
  DOMAIN: Amino acid sequence of heavy chain variable region of huB7VH2
EIQLVQSGSELKKPGASVKVSCKTSGYTFTNYGMNWVRQAPGQGLEWMGWINTYTGEPTYADDFKGRFVFSLETSVSTAYLQISSLKAEDTAVYYCARGDSFTTEILRNWYFDVWGQGTTVTVSS

SEQ ID NO: 46 - protein, 125 aa, Artificial Sequence
  DOMAIN: Amino acid sequence of heavy chain variable region of huB7VH3
EIQLVQSGSELKKPGASVKVSCKTSGYTFTNYGMNWVRQAPGQGLKWMGWINTYTGEPTYADDFKGRFVFSLETSVSTAYLQINSLKAEDTAVYYCARGDSFTTEILRNWYFDVWGQGTTVTVSS

SEQ ID NO: 47 - protein, 107 aa, Artificial Sequence
  DOMAIN: Amino acid sequence of light chain variable region of huB7VL1
DIQMTQSPSSLSASVGDRVTITCGASENIYGALNWYQQKPGKVPKLLIYGATNLADGVPSRFSGSGSGTDFTLTISSLQPEDVATYYCQNVLSTPWTFGGGTKVEIK

SEQ ID NO: 48 - protein, 107 aa, Artificial Sequence
  DOMAIN: Amino acid sequence of light chain variable region of huB7VL2
DIQMTQSPSSLSASVGDRVTITCGASENIYGALNWYQQKPGKVPKLLIYGATNLADGVPSRFSGSGSGRDYTLTISSLQPEDVATYYCQNVLSTPWTFGGGTKVEIK

SEQ ID NO: 49 - protein, 107 aa, Artificial Sequence
  DOMAIN: Amino acid sequence of light chain variable region of huB7VL3
DIQMTQSPSSLSASVGDRVTITCGASENIYGALNWYQQKPGKSPKLLIYGATNLADGVPSRFSGSGSGRDYTLTISSLQPEDVATYYCQNVLSTPWTFGGGTKVEIK

SEQ ID NO: 50 - protein, 107 aa, Artificial Sequence
  DOMAIN: Amino acid sequence of light chain variable region of huB7VL4
DIQMTQSPSSLSASVGDRVTITCGASENIYGALNWYQRKPGKSPKLLIYGATNLADGVPSRFSGSGSGRQYTLTISSLQPEDVATYYCQNVLSTPWTFGGGTKVEIK

SEQ ID NO: 51 - protein, 125 aa, Artificial Sequence
  DOMAIN: Amino acid sequence of heavy chain variable region of huB7VH1-1
EVQLVQSGSELKKPGASVKVSCKASGYTFTNYGMNWVRQAPGQGLEWMGWINTYTGEPTYADEFKGRFVFSLDTSVSTAYLQISSLKAEDTAVYYCARGDSFTTEILRNWYFDVWGQGTTVTVSS

SEQ ID NO: 52 - protein, 125 aa, Artificial Sequence
  DOMAIN: Amino acid sequence of heavy chain variable region of huB7VH2-1
EIQLVQSGSELKKPGASVKVSCKTSGYTFTNYGMNWVRQAPGQGLEWMGWINTYTGEPTYADEFKGRFVFSLETSVSTAYLQISSLKAEDTAVYYCARGDSFTTEILRNWYFDVWGQGTTVTVSS

SEQ ID NO: 53 - protein, 125 aa, Artificial Sequence
  DOMAIN: Amino acid sequence of heavy chain variable region of huB7VH3-1
EIQLVQSGSELKKPGASVKVSCKTSGYTFTNYGMNWVRQAPGQGLKWMGWINTYTGEPTYADEFKGRFVFSLETSVSTAYLQINSLKAEDTAVYYCARGDSFTTEILRNWYFDVWGQGTTVTVSS

SEQ ID NO: 54 - protein, 17 aa, Artificial Sequence
  DOMAIN: Amino acid sequence of HCDR2 mutant of B7
WINTYTGEPTYADEFKG

SEQ ID NO: 55 - protein, 120 aa, Artificial Sequence
  DOMAIN: Amino acid sequence of heavy chain variable region of huF4VH1
EVQLVQSGAEVKKPGSSVKVSCKASGGTFSRYNMHWVRQAPGQGLEWMGAIFPGNGETSYNQNFKGRVTITADKSTSTAYMELSSLRSEDTAVYYCARNSYYDYAWFTYWGQGTLVTVSS

SEQ ID NO: 56 - protein, 120 aa, Artificial Sequence
  DOMAIN: Amino acid sequence of heavy chain variable region of huF4VH2
EVQLVQSGAEVKKPGSSVKVSCKASGDTFPRYNMHWVRQAPGQGLEWMGAIFPGNGETSYNQNFKGRVTITADKSTSTAYMELSSLRSEDTAVYYCARNSYYDYAWFTYWGQGTLVTVSS

SEQ ID NO: 57 - protein, 120 aa, Artificial Sequence
  DOMAIN: Amino acid sequence of heavy chain variable region of huF4VH3
EVQLVQSGAEVKKPGSSVKVSCKASGDTFPRYNMHWVRQAPGQGLEWMGAIFPGNGETSYNQNFKGRVTLTADKSTSTAYMELSSLRSEDTAVYYCARNSYYDYAWFTYWGQGTLVTVSS

SEQ ID NO: 58 - protein, 120 aa, Artificial Sequence
  DOMAIN: Amino acid sequence of heavy chain variable region of huF4VH4
EVQLVQSGAEVKKPGSSVKVSCKASGDTFPRYNMHWLKQAPGQGLEWMGAIFPGNGETSYNQNFKGRVTLTADKSTSTAYMELSSLRSEDTAVYYCARNSYYDYAWFTYWGQGTLVTVSS

SEQ ID NO: 59 - protein, 120 aa, Artificial Sequence
  DOMAIN: Amino acid sequence of heavy chain variable region of huF4VH5
EVQLVQSGAEVKKPGSSVKVSCKASGDTFPRYNMHWLKQAPGQGLEWMGAIFPGNGETSYNQNFKGKVTLTADKSTSTAYMELNSLRSEDTAVYYCARNSYYDYAWFTYWGQGTLVTVSS

SEQ ID NO: 60 - protein, 120 aa, Artificial Sequence
  DOMAIN: Amino acid sequence of heavy chain variable region of huF4VH6
EVQLVQSGAEVKKPGSSVKVSCKASGDTFPRYNMHWLKQAPGQGLEWIGAIFPGNGETSYNQNFKGKATLTADKSTSTAYMELNSLRSEDTAVYYCARNSYYDYAWFTYWGQGTLVTVSS

SEQ ID NO: 61 - protein, 111 aa, Artificial Sequence
  DOMAIN: Amino acid sequence of light chain variable region of huF4VL1
DIVMTQSPDSLAVSLGERATINCRASKSVSSSGYSFMHWYQQKPGQPPKLLIYLASNLESGVPDRFSGSGSGTDFTLTISSLQAEDVAVYYCQHSREFPPTFGQGTKLEIK

SEQ ID NO: 62 - protein, 111 aa, Artificial Sequence
  DOMAIN: Amino acid sequence of light chain variable region of huF4VL2
DIVMTQSPDSLAVSLGERATINCRASKSVSSSGYSFMHWYQQKPGQPPKLLISLASNLESGVPDRFSGSGSGTDFTLTISSLQAEDVAVYYCQHSREFPPTFGQGTKLEIK

SEQ ID NO: 63 - protein, 120 aa, Artificial Sequence
  DOMAIN: Amino acid sequence of heavy chain variable region of huF4VH1-1
EVQLVQSGAEVKKPGSSVKVSCKASGGTFSRYNMHWVRQAPGQGLEWMGAIFPGTGETSYNQNFKGRVTITADKSTSTAYMELSSLRSEDTAVYYCARNSYYDYAWFTYWGQGTLVTVSS

SEQ ID NO: 64 - protein, 120 aa, Artificial Sequence
  DOMAIN: Amino acid sequence of heavy chain variable region of huF4VH2-1
EVQLVQSGAEVKKPGSSVKVSCKASGDTFPRYNMHWVRQAPGQGLEWMGAIFPGTGETSYNQNFKGRVTITADKSTSTAYMELSSLRSEDTAVYYCARNSYYDYAWFTYWGQGTLVTVSS

SEQ ID NO: 65 - protein, 120 aa, Artificial Sequence
  DOMAIN: Amino acid sequence of heavy chain variable region of huF4VH3-1
EVQLVQSGAEVKKPGSSVKVSCKASGDTFPRYNMHWVRQAPGQGLEWMGAIFPGTGETSYNQNFKGRVTLTADKSTSTAYMELSSLRSEDTAVYYCARNSYYDYAWFTYWGQGTLVTVSS

SEQ ID NO: 66 - protein, 120 aa, Artificial Sequence
  DOMAIN: Amino acid sequence of heavy chain variable region of huF4VH4-1
EVQLVQSGAEVKKPGSSVKVSCKASGDTFPRYNMHWLKQAPGQGLEWMGAIFPGTGETSYNQNFKGRVTLTADKSTSTAYMELSSLRSEDTAVYYCARNSYYDYAWFTYWGQGTLVTVSS

SEQ ID NO: 67 - protein, 120 aa, Artificial Sequence
  DOMAIN: Amino acid sequence of heavy chain variable region of huF4VH5-1
EVQLVQSGAEVKKPGSSVKVSCKASGDTFPRYNMHWLKQAPGQGLEWMGAIFPGTGETSYNQNFKGKVTLTADKSTSTAYMELNSLRSEDTAVYYCARNSYYDYAWFTYWGQGTLVTVSS

SEQ ID NO: 68 - protein, 120 aa, Artificial Sequence
  DOMAIN: Amino acid sequence of heavy chain variable region of huF4VH6-1
EVQLVQSGAEVKKPGSSVKVSCKASGDTFPRYNMHWLKQAPGQGLEWIGAIFPGTGETSYNQNFKGKATLTADKSTSTAYMELNSLRSEDTAVYYCARNSYYDYAWFTYWGQGTLVTVSS

SEQ ID NO: 69 - protein, 111 aa, Artificial Sequence
  DOMAIN: Amino acid sequence of light chain variable region of huF4VL1-1
DIVMTQSPDSLAVSLGERATINCRASKSVSSSGYSFMHWYQQKPGQPPKLLIYLADNLESGVPDRFSGSGSGTDFTLTISSLQAEDVAVYYCQHSREFPPTFGQGTKLEIK

SEQ ID NO: 70 - protein, 111 aa, Artificial Sequence
  DOMAIN: Amino acid sequence of light chain variable region of huF4VL2-1
DIVMTQSPDSLAVSLGERATINCRASKSVSSSGYSFMHWYQQKPGQPPKLLISLADNLESGVPDRFSGSGSGTDFTLTISSLQAEDVAVYYCQHSREFPPTFGQGTKLEIK

SEQ ID NO: 71 - protein, 17 aa, Artificial Sequence
  DOMAIN: Amino acid sequence of HCDR2 mutant of F4
AIFPGTGETSYNQNFKG

SEQ ID NO: 72 - protein, 330 aa, Artificial Sequence [sequence omitted]

SEQ ID NO: 73 - protein, 107 aa, Artificial Sequence [sequence omitted]

SEQ ID NO: 74 - protein, 449 aa, Artificial Sequence
  CHAIN: Heavy chain sequence of huB1010
EVQMVQSGAEVKKPGASVKVSCKASGYTFTTYNIHWVRQAPGQGLEWMGDIYPGTGDASYNQKFRDRVTMTRDTSTSTVYMELSSLRSEDTAVYYCATFSRFDGWFAYWGQGTLVTVSSASTKGPSVFPLAPSSKSTSGGTAALGCLVKDYFPEPVTVSWNSGALTSGVHTFPAVLQSSGLYSLSSVVTVPSSSLGTQTYICNVNHKPSNTKVDKKVEPKSCDKTHTCPPCPAPELLGGPSVFLFPPKPKDTLMISRTPEVTCVVVDVSHEDPEVKFNWYVDGVEVHNAKTKPREEQYNSTYRVVSVLTVLHQDWLNGKEYKCKVSNKALPAPIEKTISKAKGQPREPQVYTLPPSRDELTKNQVSLTCLVKGFYPSDIAVEWESNGQPENNYKTTPPVLDSDGSFFLYSKLTVDKSRWQQGNVFSCSVMHEALHNHYTQKSLSLSPGK

SEQ ID NO: 75 - protein, 218 aa, Artificial Sequence
  CHAIN: Light chain sequence of huB1010
DIVMTQSPDSLAVSLGERATINCRASRSVSTSGYSYMHWYQQKPGQPPKLLIYLADNLESGVPDRFSGSGSGTDFTLTISSLQAEDVAVYYCQHSRELPYTFGGGTKVEIKRTVAAPSVFIFPPSDEQLKSGTASVVCLLNNFYPREAKVQWKVDNALQSGNSQESVTEQDSKDSTYSLSSTLTLSKADYEKHKVYACEVTHQGLSSPVTKSFNRGEC

SEQ ID NO: 76 - protein, 455 aa, Artificial Sequence
  CHAIN: Heavy chain sequence of huB7002
EVQLVQSGSELKKPGASVKVSCKASGYTFTNYGMNWVRQAPGQGLEWMGWINTYTGEPTYADEFKGRFVFSLDTSVSTAYLQISSLKAEDTAVYYCARGDSFTTEILRNWYFDVWGQGTTVTVSSASTKGPSVFPLAPSSKSTSGGTAALGCLVKDYFPEPVTVSWNSGALTSGVHTFPAVLQSSGLYSLSSVVTVPSSSLGTQTYICNVNHKPSNTKVDKKVEPKSCDKTHTCPPCPAPELLGGPSVFLFPPKPKDTLMISRTPEVTCVVVDVSHEDPEVKFNWYVDGVEVHNAKTKPREEQYNSTYRVVSVLTVLHQDWLNGKEYKCKVSNKALPAPIEKTISKAKGQPREPQVYTLPPSRDELTKNQVSLTCLVKGFYPSDIAVEWESNGQPENNYKTTPPVLDSDGSFFLYSKLTVDKSRWQQGNVFSCSVMHEALHNHYTQKSLSLSPGK

SEQ ID NO: 77 - protein, 214 aa, Artificial Sequence
  CHAIN: Light chain sequence of huB7002
DIQMTQSPSSLSASVGDRVTITCGASENIYGALNWYQQKPGKVPKLLIYGATNLADGVPSRFSGSGSGTDFTLTISSLQPEDVATYYCQNVLSTPWTFGGGTKVEIKRTVAAPSVFIFPPSDEQLKSGTASVVCLLNNFYPREAKVQWKVDNALQSGNSQESVTEQDSKDSTYSLSSTLTLSKADYEKHKVYACEVTHQGLSSPVTKSFNRGEC

SEQ ID NO: 78 - protein, 450 aa, Artificial Sequence
  CHAIN: Heavy chain sequence of huF4011
EVQLVQSGAEVKKPGSSVKVSCKASGDTFPRYNMHWVRQAPGQGLEWMGAIFPGTGETSYNQNFKGRVTLTADKSTSTAYMELSSLRSEDTAVYYCARNSYYDYAWFTYWGQGTLVTVSSASTKGPSVFPLAPSSKSTSGGTAALGCLVKDYFPEPVTVSWNSGALTSGVHTFPAVLQSSGLYSLSSVVTVPSSSLGTQTYICNVNHKPSNTKVDKKVEPKSCDKTHTCPPCPAPELLGGPSVFLFPPKPKDTLMISRTPEVTCVVVDVSHEDPEVKFNWYVDGVEVHNAKTKPREEQYNSTYRVVSVLTVLHQDWLNGKEYKCKVSNKALPAPIEKTISKAKGQPREPQVYTLPPSRDELTKNQVSLTCLVKGFYPSDIAVEWESNGQPENNYKTTPPVLDSDGSFFLYSKLTVDKSRWQQGNVFSCSVMHEALHNHYTQKSLSLSPGK

SEQ ID NO: 79 - protein, 218 aa, Artificial Sequence
  CHAIN: Light chain sequence of huF4011
DIVMTQSPDSLAVSLGERATINCRASKSVSSSGYSFMHWYQQKPGQPPKLLISLADNLESGVPDRFSGSGSGTDFTLTISSLQAEDVAVYYCQHSREFPPTFGQGTKLEIKRTVAAPSVFIFPPSDEQLKSGTASVVCLLNNFYPREAKVQWKVDNALQSGNSQESVTEQDSKDSTYSLSSTLTLSKADYEKHKVYACEVTHQGLSSPVTKSFNRGEC

SEQ ID NO: 80 - protein, 452 aa, Artificial Sequence
  CHAIN: Heavy chain sequence of 41D12
EVQLVESGGGLVQPGGSLRLSCAASGFTFSVYYMNWVRQAPGKGLEWVSDINNEGGTTYYADSVKGRFTISRDNSKNSLYLQMNSLRAEDTAVYYCARDAGYSNHVPIFDSWGQGTLVTVSSASTKGPSVFPLAPSSKSTSGGTAALGCLVKDYFPEPVTVSWNSGALTSGVHTFPAVLQSSGLYSLSSVVTVPSSSLGTQTYICNVNHKPSNTKVDKKVEPKSCDKTHTCPPCPAPELLGGPSVFLFPPKPKDTLMISRTPEVTCVVVDVSHEDPEVKFNWYVDGVEVHNAKTKPREEQYNSTYRVVSVLTVLHQDWLNGKEYKCKVSNKALPAPIEKTISKAKGQPREPQVYTLPPSRDELTKNQVSLTCLVKGFYPSDIAVEWESNGQPENNYKTTPPVLDSDGSFFLYSKLTVDKSRWQQGNVFSCSVMHEALHNHYTQKSLSLSPGK

SEQ ID NO: 81 - protein, 216 aa, Artificial Sequence
  CHAIN: Light chain sequence of 41D12
QAVVTQEPSLTVSPGGTVTLTCGLKSGSVTSDNFPTWYQQTPGQAPRLLIYNTNTRHSGVPDRFSGSILGNKAALTITGAQADDEAEYFCALFISNPSVEFGGGTQLTVLGQPKAAPSVTLFPPSSEELQANKATLVCLISDFYPGAVTVAWKADSSPVKAGVETTTPSKQSNNKYAASSYLSLTPEQWKSHRSYSCQVTHEGSTVEKTVAPTECS

SEQ ID NO: 82 - protein, 388 aa, Artificial Sequence
  PEPTIDE: Sequence of fusion protein of monkey CD70 protein extracellular domain and Human-IgG1-Fc
QRLSRAQQQLPLESLGWDIAELQLNHTGPQQDPRLYWQGGPALGRSFLHGPELDKGQLRIRRDGIYMVHIQVTLAICSSTSTSRHHHPTTLAVGICSPASRSISLLRLSFHQGCTIASQRLTPLARGDTLCTNLTGTLLPSRNTDETFFGVQWVRPEPKSSDKTHTCPPCPAPELLGGPSVFLFPPKPKDTLMISRTPEVTCVVVDVSHEDPEVKFNWYVDGVEVHNAKTKPREEQYNSTYRVVSVLTVLHQDWLNGKEYKCKVSNKALPAPIEKTISKAKGQPREPQVYTLPPSRDELTKNQVSLTCLVKGFYPSDIAVEWESNGQPENNYKTTPPVLDSDGSFFLYSKLTVDKSRWQQGNVFSCSVMHEALHNHYTQKSLSLSPGK

SEQ ID NO: 83 - protein, 383 aa, Artificial Sequence
  PEPTIDE: Sequence of fusion protein of murine CD70 protein extracellular domain and Human-IgG1-Fc
SKQQQRLLEHPEPHTAELQLNLTVPRKDPTLRWGAGPALGRSFTHGPELEEGHLRIHQDGLYRLHIQVTLANCSSPGSTLQHRATLAVGICSPAAHGISLLRGRFGQDCTVALQRLTYLVHGDVLCTNLTLPLLPSRNADETFFGVQWICPEPKSSDKTHTCPPCPAPELLGGPSVFLFPPKPKDTLMISRTPEVTCVVVDVSHEDPEVKFNWYVDGVEVHNAKTKPREEQYNSTYRVVSVLTVLHQDWLNGKEYKCKVSNKALPAPIEKTISKAKGQPREPQVYTLPPSRDELTKNQVSLTCLVKGFYPSDIAVEWESNGQPENNYKTTPPVLDSDGSFFLYSKLTVDKSRWQQGNVFSCSVMHEALHNHYTQKSLSLSPGK

SEQ ID NO: 84 - protein, 414 aa, Artificial Sequence
  PEPTIDE: Sequence of fusion protein of human CD27 and Human-IgG1-Fc
ATPAPKSCPERHYWAQGKLCCQMCEPGTFLVKDCDQHRKAAQCDPCIPGVSFSPDHHTRPHCESCRHCNSGLLVRNCTITANAECACRNGWQCRDKECTECDPLPNPSLTARSSQALSPHPQPTHLPYVSEMLEARTAGHMQTLADFRQLPARTLSTHWPPQRSLCSSDFIRGGGGSGGGGSEPKSSDKTHTCPPCPAPELLGGPSVFLFPPKPKDTLMISRTPEVTCVVVDVSHEDPEVKFNWYVDGVEVHNAKTKPREEQYNSTYRVVSVLTVLHQDWLNGKEYKCKVSNKALPAPIEKTISKAKGQPREPQVYTLPPSRDELTKNQVSLTCLVKGFYPSDIAVEWESNGQPENNYKTTPPVLDSDGSFFLYSKLTVDKSRWQQGNVFSCSVMHEALHNHYTQKSLSLSPGK